European Patent Application EP 4 545 965 A2, published April 30, 2025. Title: Methods and compositions for proximity ligation. Applicant: Dovetail Genomics, LLC. Application EP. The sequence listing filed with the application follows.

SEQUENCE LISTING (38 sequences)

SEQ ID NO: 1 - DNA, 37 bp, synthetic construct
  misc_feature 1..37: note = Description of Artificial Sequence: Synthetic oligonucleotide
  source 1..37: mol_type = other DNA
gtgccagggcgtgcccttgggctccccgggcgcgatc

SEQ ID NO: 2 - DNA, 10 bp, synthetic construct
  misc_feature 1..10: note = Description of Artificial Sequence: Synthetic oligonucleotide
  source 1..10: mol_type = other DNA
gcccttgggc

SEQ ID NO: 3 - DNA, 34 bp, synthetic construct
  misc_feature 1..34: note = Description of Artificial Sequence: Synthetic oligonucleotide
  source 1..34: mol_type = other DNA
cgcgcccggggagcccaagggcacgccctggcac

SEQ ID NO: 4 - DNA, 10 bp, synthetic construct
  misc_feature 1..10: note = Description of Artificial Sequence: Synthetic oligonucleotide
  source 1..10: mol_type = other DNA
gcccaagggc

SEQ ID NO: 5 - DNA, 39 bp, synthetic construct
  misc_feature 1..39: note = Description of Artificial Sequence: Synthetic oligonucleotide
  source 1..39: mol_type = other DNA
gtgccagggcgtgcccttgggctccccgggcgcgtcccc

SEQ ID NO: 6 - DNA, 39 bp, synthetic construct
  misc_feature 1..39: note = Description of Artificial Sequence: Synthetic oligonucleotide
  source 1..39: mol_type = other DNA
ggggacgcgcccggggagcccaagggcacgccctggcac

SEQ ID NO: 7 - DNA, 99 bp, synthetic construct
  misc_feature 1..99: note = Description of Artificial Sequence: Synthetic oligonucleotide
  source 1..99: mol_type = other DNA
ggagccccaactggggtaacctttgagttctctcagttggggaccatggagatcaccccaactgagagaactcaaaggttaccccagttggggcactac

SEQ ID NO: 8 - DNA, 10 bp, synthetic construct
  misc_feature 1..10: note = Description of Artificial Sequence: Synthetic oligonucleotide
  source 1..10: mol_type = other DNA
acctttgagt

SEQ ID NO: 9 - DNA, 10 bp, synthetic construct
  misc_feature 1..10: note = Description of Artificial Sequence: Synthetic oligonucleotide
  source 1..10: mol_type = other DNA
catggagatc

SEQ ID NO: 10 - DNA, 91 bp, synthetic construct
  misc_feature 1..91: note = Description of Artificial Sequence: Synthetic oligonucleotide
  source 1..91: mol_type = other DNA
ggagccccaactggggtaacctttgagttctctcagttggggaccatggagatcaccccaactgagagaactcaagggcacgccctggcac

SEQ ID NO: 11 - DNA, 85 bp, synthetic construct
  misc_feature 1..85: note = Description of Artificial Sequence: Synthetic oligonucleotide
  source 1..85: mol_type = other DNA
gtgccagggcgtgcccttgagttctctcagttggggaccatggagatcaccccaactgagagaactcaagggcacgccctggcac

SEQ ID NO: 12 - DNA, 10 bp, synthetic construct
  misc_feature 1..10: note = Description of Artificial Sequence: Synthetic oligonucleotide
  source 1..10: mol_type = other DNA
gcccttgagt

SEQ ID NO: 13 - DNA, 10 bp, synthetic construct
  misc_feature 1..10: note = Description of Artificial Sequence: Synthetic oligonucleotide
  source 1..10: mol_type = other DNA
actcaagggc

SEQ ID NO: 14 - DNA, 34 bp, synthetic construct
  misc_feature 1..34: note = Description of Artificial Sequence: Synthetic oligonucleotide
  source 1..34: mol_type = other DNA
gtgccagggcgtgcccttgggctccccgggcgcg

SEQ ID NO: 15 - DNA, 33 bp, synthetic construct
  misc_feature 1..33: note = Description of Artificial Sequence: Synthetic oligonucleotide
  source 1..33: mol_type = other DNA
gatcggaagagcacacgtctgaactccagtcac

SEQ ID NO: 16 - DNA, 32 bp, synthetic construct
  misc_feature 1..32: note = Description of Artificial Sequence: Synthetic oligonucleotide
  source 1..32: mol_type = other DNA
acactctttccctacacgacgctcttccgatc

SEQ ID NO: 17 - skipped

SEQ ID NO: 18 - DNA, 67 bp, synthetic construct
  misc_feature 1..67: note = Description of Artificial Sequence: Synthetic oligonucleotide
  source 1..67: mol_type = other DNA
ctagccttctcgcagcacatccctttctcacacgcgcccggggagcccaagggcacgccctggcact

SEQ ID NO: 19 - skipped

SEQ ID NO: 20 - DNA, 67 bp, synthetic construct
  misc_feature 1..67: note = Description of Artificial Sequence: Synthetic oligonucleotide
  source 1..67: mol_type = other DNA
gtgccagggcgtgcccttgggctccccgggcgcggatcggaagagcacacgtctgaactccagtcac

SEQ ID NO: 21-22 - skipped (2 entries)

SEQ ID NO: 23 - DNA, 25 bp, synthetic construct
  misc_feature 1..25: note = Description of Artificial Sequence: Synthetic oligonucleotide
  misc_feature 1..6: note = n = a, c, t, g, unknown or other
  misc_feature 10..12: note = n = a, c, t, g, unknown or other
  misc_feature 18..20: note = n = a, c, t, g, unknown or other
  source 1..25: mol_type = other DNA
nnnnnnatgnnntcaaannntcatg

SEQ ID NO: 24 - DNA, 22 bp, synthetic construct
  misc_feature 1..22: note = Description of Artificial Sequence: Synthetic oligonucleotide
  misc_feature 3..5: note = n = a, c, t, g, unknown or other
  misc_feature 11..13: note = n = a, c, t, g, unknown or other
  misc_feature 17..22: note = n = a, c, t, g, unknown or other
  source 1..22: mol_type = other DNA
gannntttgannncatnnnnnn

SEQ ID NO: 25 - DNA, 35 bp, synthetic construct
  misc_feature 1..35: note = Description of Artificial Sequence: Synthetic oligonucleotide
  misc_feature 1..6: note = n = a, c, t, g, unknown or other
  misc_feature 10..12: note = n = a, c, t, g, unknown or other
  misc_feature 18..20: note = n = a, c, t, g, unknown or other
  misc_feature 27..29: note = n = a, c, t, g, unknown or other
  source 1..35: mol_type = other DNA
nnnnnnatgnnntcaaannntcatgcnnnatgatc

SEQ ID NO: 26 - DNA, 31 bp, synthetic construct
  misc_feature 1..31: note = Description of Artificial Sequence: Synthetic oligonucleotide
  misc_feature 3..5: note = n = a, c, t, g, unknown or other
  misc_feature 12..14: note = n = a, c, t, g, unknown or other
  misc_feature 20..22: note = n = a, c, t, g, unknown or other
  misc_feature 26..31: note = n = a, c, t, g, unknown or other
  source 1..31: mol_type = other DNA
atnnngcatgannntttgannncatnnnnnn

SEQ ID NO: 27 - DNA, 66 bp, synthetic construct
  misc_feature 1..66: note = Description of Artificial Sequence: Synthetic oligonucleotide
  misc_feature 1..6: note = n = a, c, t, g, unknown or other
  misc_feature 10..12: note = n = a, c, t, g, unknown or other
  misc_feature 18..20: note = n = a, c, t, g, unknown or other
  misc_feature 27..29: note = n = a, c, t, g, unknown or other
  misc_feature 38..40: note = n = a, c, t, g, unknown or other
  misc_feature 47..49: note = n = a, c, t, g, unknown or other
  misc_feature 55..57: note = n = a, c, t, g, unknown or other
  misc_feature 61..66: note = n = a, c, t, g, unknown or other
  source 1..66: mol_type = other DNA
nnnnnnatgnnntcaaannntcatgcnnnatgatcatnnngcatgannntttgannncatnnnnnn

SEQ ID NO: 28 - DNA, 37 bp, synthetic construct
  misc_feature 1..37: note = Description of Artificial Sequence: Synthetic oligonucleotide
  source 1..37: mol_type = other DNA
agtgccagggcgtgcccttgagttctctcagttgggg

SEQ ID NO: 29 - DNA, 28 bp, synthetic construct
  misc_feature 1..28: note = Description of Artificial Sequence: Synthetic oligonucleotide
  misc_feature 3..5: note = n = a, c, t, g, unknown or other
  misc_feature 11..13: note = n = a, c, t, g, unknown or other
  misc_feature 20..22: note = n = a, c, t, g, unknown or other
  source 1..28: mol_type = other DNA
tgnnntcaaannntcatgcnnnatgatc

SEQ ID NO: 30 - DNA, 25 bp, synthetic construct
  misc_feature 1..25: note = Description of Artificial Sequence: Synthetic oligonucleotide
  misc_feature 3..5: note = n = a, c, t, g, unknown or other
  misc_feature 12..14: note = n = a, c, t, g, unknown or other
  misc_feature 20..22: note = n = a, c, t, g, unknown or other
  source 1..25: mol_type = other DNA
atnnngcatgannntttgannncat

SEQ ID NO: 31 - DNA, 38 bp, synthetic construct
  misc_feature 1..38: note = Description of Artificial Sequence: Synthetic oligonucleotide
  source 1..38: mol_type = other DNA
agtgccagggcgtgcccttgggctccccgggcgcgatc

SEQ ID NO: 32 - DNA, 35 bp, synthetic construct
  misc_feature 1..35: note = Description of Artificial Sequence: Synthetic oligonucleotide
  source 1..35: mol_type = other DNA
cgcgcccggggagcccaagggcacgccctggcact

SEQ ID NO: 33 - DNA, 40 bp, synthetic construct
  misc_feature 1..40: note = Description of Artificial Sequence: Synthetic oligonucleotide
  source 1..40: mol_type = other DNA
agtgccagggcgtgcccttgggctccccgggcgcgtcccc

SEQ ID NO: 34 - DNA, 40 bp, synthetic construct
  misc_feature 1..40: note = Description of Artificial Sequence: Synthetic oligonucleotide
  source 1..40: mol_type = other DNA
ggggacgcgcccggggagcccaagggcacgccctggcact

SEQ ID NO: 35 - DNA, 92 bp, synthetic construct
  misc_feature 1..92: note = Description of Artificial Sequence: Synthetic oligonucleotide
  source 1..92: mol_type = other DNA
ggagccccaactggggtaacctttgagttctctcagttggggaccatggagatcaccccaactgagagaactcaagggcacgccctggcact

SEQ ID NO: 36 - DNA, 41 bp, synthetic construct
  misc_feature 1..41: note = Description of Artificial Sequence: Synthetic oligonucleotide
  source 1..41: mol_type = other DNA
ccccaactgagagaactcaaaggttacccagttggggctcc

SEQ ID NO: 37 - DNA, 87 bp, synthetic construct
  misc_feature 1..87: note = Description of Artificial Sequence: Synthetic oligonucleotide
  source 1..87: mol_type = other DNA
agtgccagggcgtgcccttgagttctctcagttggggaccatggagatcaccccaactgagagaactcaagggcacgccctggcact

SEQ ID NO: 38 - DNA, 37 bp, synthetic construct
  misc_feature 1..37: note = Description of Artificial Sequence: Synthetic oligonucleotide
  source 1..37: mol_type = other DNA
ccccaactgagagaactcaagggcacgccctggcact